European Patent Application EP 4 317 411 A1, published February 7, 2024. Title: LACTOBACILLUS RHAMNOSUS, FERMENT LYSATE FOR REGULATING SKIN MICROECOLOGY, PREPARATION METHOD, AND APPLICATION. Applicant: Bloomage Biotechnology Corporation Limited. The sequence listing filed with the application follows.

SEQUENCE LISTING (3 sequences)

SEQ ID NO: 1 - DNA, 20 bp, Artificial sequence
  Description of artificial sequence: Artificially synthesized sequence
agagtttgatcmtggctcag

SEQ ID NO: 2 - DNA, 19 bp, Artificial sequence
  Description of artificial sequence: Artificially synthesized sequence
ggttaccttgttacgactt

SEQ ID NO: 3 - DNA, 1517 bp, Lactobacillus rhamnosus
tttgatcatggctcaggatgaatactggcggcgtgcctaatacatgcaagtcgaacgagttctgattattgaaaggtgcttgcatcttgatttaattttgaacgagtggcggacgggtgagtaacacgtgggtaacctgcccttaagtgggggataacatttggaaacagatgctaataccgcataaatccaagaaccgcatggttcttggctgaaagatggcgtaagctatcgcttttggatggacccgcggcgtattagctagttggtgaggtaacggctcaccaaggcaatgatacgtagccgaactgagaggttgatcggccacattgggactgagacacggcccaaactcctacgggaggcagcagtagggaatcttccacaatggacgcaagtctgatggagcaacgccgcgtgagtgaagaaggctttcgggtcgtaaaactctgttgttggagaagaatggtcggcagagtaactgttgtcggcgtgacggtatccaaccagaaagccacggctaactacgtgccagcagccgcggtaatacgtaggtggcaagcgttatccggatttattgggcgtaaagcgagcgcaggcggttttttaagtctgatgtgaaagccctcggcttaaccgaggaagtgcatcggaaactgggaaacttgagtgcagaagaggacagtggaactccatgtgtagcggtgaaatgcgtagatatatggaagaacaccagtggcgaaggcggctgtctggtctgtaactgacgctgaggctcgaaagcatgggtagcgaacaggattagataccctggtagtccatgccgtaaacgatgaatgctaggtgttggagggtttccgcccttcagtgccgcagctaacgcattaagcattccgcctggggagtacgaccgcaaggttgaaactcaaaggaattgacgggggcccgcacaagcggtggagcatgtggtttaattcgaagcaacgcgaagaaccttaccaggtcttgacatcttttgatcacctgagagatcaggtttccccttcgggggcaaaatgacaggtggtgcatggttgtcgtcagctcgtgtcgtgagatgttgggttaagtcccgcaacgagcgcaacccttatgactagttgccagcatttagttgggcactctagtaagactgccggtgacaaaccggaggaaggtggggatgacgtcaaatcatcatgccccttatgacctgggctacacacgtgctacaatggatggtacaacgagttgcgagaccgcgaggtcaagctaatctcttaaagccattctcagttcggactgtaggctgcaactcgcctacacgaagtcggaatcgctagtaatcgcggatcagcacgccgcggtgaatacgttcccgggccttgtacacaccgcccgtcacaccatgagagtttgtaacacccgaagccggtggcgtaacccttttagggagcgagccgtctaaggtgggacaaatgattagggtgaagtcgtaa